European Patent Application EP 4 640 827 A1, published October 29, 2025. Title: Novel recombinant TET3-enzymes. Applicant: Ludwig-Maximilians-Universitaet Muenchen; Koerperschaft des oeffentlichen Rechts. The sequence listing filed with the application follows.

SEQUENCE LISTING (21 sequences)

SEQ ID NO: 1 - protein, 1668 aa, Mus musculus
  source 1..1668: note = Mouse (mus musculus) TET3-enzyme (short isoform; Uniprot No A0A5K1VVP6)
MDSGPVYHGDSRQLSTSGAPVNGAREPAGPGLLGAAGPWRVDQKPDWEAASGPTHAARLEDAHDLVAFSAVAEAVSSYGALSTRLYETFNREMSREAGSNGRGPRPESCSEGSEDLDTLQTALALARHGMKPPNCTCDGPECPDFLEWLEGKIKSMAMEGGQGRPRLPGALPPSEAGLPAPSTRPPLLSSEVPQVPPLEGLPLSQSALSIAKEKNISLQTAIAIEALTQLSSALPQPSHSTSQASCPLPEALSPSAPFRSPQSYLRAPSWPVVPPEEHPSFAPDSPAFPPATPRPEFSEAWGTDTPPATPRNSWPVPRPSPDPMAELEQLLGSASDYIQSVFKRPEALPTKPKVKVEAPSSSPAPVPSPISQREAPLLSSEPDTHQKAQTALQQHLHHKRNLFLEQAQDASFPTSTEPQAPGWWAPPGSPAPRPPDKPPKEKKKKPPTPAGGPVGAEKTTPGIKTSVRKPIQIKKSRSRDMQPLFLPVRQIVLEGLKPQASEGQAPLPAQLSVPPPASQGAASQSCATPLTPEPSLALFAPSPSGDSLLPPTQEMRSPSPMVALQSGSTGGPLPPADDKLEELIRQFEAEFGDSFGLPGPPSVPIQEPENQSTCLPAPESPFATRSPKKIKIESSGAVTVLSTTCFHSEEGGQEATPTKAENPLTPTLSGFLESPLKYLDTPTKSLLDTPAKKAQSEFPTCDCVEQIVEKDEGPYYTHLGSGPTVASIRELMEDRYGEKGKAIRIEKVIYTGKEGKSSRGCPIAKWVIRRHTLEEKLLCLVRHRAGHHCQNAVIVILILAWEGIPRSLGDTLYQELTDTLRKYGNPTSRRCGLNDDRTCACQGKDPNTCGASFSFGCSWSMYFNGCKYARSKTPRKFRLTGDNPKEEEVLRNSFQDLATEVAPLYKRLAPQAYQNQVTNEDVAIDCRLGLKEGRPFSGVTACMDFCAHAHKDQHNLYNGCTVVCTLTKEDNRCVGQIPEDEQLHVLPLYKMASTDEFGSEENQNAKVSSGAIQVLTAFPREVRRLPEPAKSCRQRQLEARKAAAEKKKLQKEKLSTPEKIKQEALELAGVTTDPGLSLKGGLSQQSLKPSLKVEPQNHFSSFKYSGNAVVESYSVLGSCRPSDPYSMSSVYSYHSRYAQPGLASVNGFHSKYTLPSFGYYGFPSSNPVFPSQFLGPSAWGHGGSGGSFEKKPDLHALHNSLNPAYGGAEFAELPGQAVATDNHHPIPHHQQPAYPGPKEYLLPKVPQLHPASRDPSPFAQSSSCYNRSIKQEPIDPLTQAESIPRDSAKMSRTPLPEASQNGGPSHLWGQYSGGPSMSPKRTNSVGGNWGVFPPGESPTIVPDKLNSFGASCLTPSHFPESQWGLFTGEGQQSAPHAGARLRGKPWSPCKFGNGTSALTGPSLTEKPWGMGTGDFNPALKGGPGFQDKLWNPVKVEEGRIPTPGANPLDKAWQAFGMPLSSNEKLFGALKSEEKLWDPFSLEEGTAEEPPSKGVVKEEKSGPTVEEDEEELWSDSEHNFLDENIGGVAVAPAHCSILIECARRELHATTPLKKPNRCHPTRISLVFYQHKNLNQPNHGLALWEAKMKQLAERARQRQEEAARLGLGQQEAKLYGKKRKWGGAMVAEPQHKEKKGAIPTRQALAMPTDSAVTVSSYAYTKVTGPYSRWI

SEQ ID NO: 2 - protein, 1803 aa, Mus musculus
  source 1..1803: note = Mouse (mus musculus) TET3-enzyme (long isoform; Uniprot No Q8BG87)
MSQFQVPLAVQPDLSGLYDFPQGQVMVGGFQGPGLPMAGSETQLRGGGDGRKKRKRCGTCDPCRRLENCGSCTSCTNRRTHQICKLRKCEVLKKKAGLLKEVEINAREGTGPWAQGATVKTGSELSPVDGPVPGQMDSGPVYHGDSRQLSTSGAPVNGAREPAGPGLLGAAGPWRVDQKPDWEAASGPTHAARLEDAHDLVAFSAVAEAVSSYGALSTRLYETFNREMSREAGSNGRGPRPESCSEGSEDLDTLQTALALARHGMKPPNCTCDGPECPDFLEWLEGKIKSMAMEGGQGRPRLPGALPPSEAGLPAPSTRPPLLSSEVPQVPPLEGLPLSQSALSIAKEKNISLQTAIAIEALTQLSSALPQPSHSTSQASCPLPEALSPSAPFRSPQSYLRAPSWPVVPPEEHPSFAPDSPAFPPATPRPEFSEAWGTDTPPATPRNSWPVPRPSPDPMAELEQLLGSASDYIQSVFKRPEALPTKPKVKVEAPSSSPAPVPSPISQREAPLLSSEPDTHQKAQTALQQHLHHKRNLFLEQAQDASFPTSTEPQAPGWWAPPGSPAPRPPDKPPKEKKKKPPTPAGGPVGAEKTTPGIKTSVRKPIQIKKSRSRDMQPLFLPVRQIVLEGLKPQASEGQAPLPAQLSVPPPASQGAASQSCATPLTPEPSLALFAPSPSGDSLLPPTQEMRSPSPMVALQSGSTGGPLPPADDKLEELIRQFEAEFGDSFGLPGPPSVPIQEPENQSTCLPAPESPFATRSPKKIKIESSGAVTVLSTTCFHSEEGGQEATPTKAENPLTPTLSGFLESPLKYLDTPTKSLLDTPAKKAQSEFPTCDCVEQIVEKDEGPYYTHLGSGPTVASIRELMEDRYGEKGKAIRIEKVIYTGKEGKSSRGCPIAKWVIRRHTLEEKLLCLVRHRAGHHCQNAVIVILILAWEGIPRSLGDTLYQELTDTLRKYGNPTSRRCGLNDDRTCACQGKDPNTCGASFSFGCSWSMYFNGCKYARSKTPRKFRLTGDNPKEEEVLRNSFQDLATEVAPLYKRLAPQAYQNQVTNEDVAIDCRLGLKEGRPFSGVTACMDFCAHAHKDQHNLYNGCTVVCTLTKEDNRCVGQIPEDEQLHVLPLYKMASTDEFGSEENQNAKVSSGAIQVLTAFPREVRRLPEPAKSCRQRQLEARKAAAEKKKLQKEKLSTPEKIKQEALELAGVTTDPGLSLKGGLSQQSLKPSLKVEPQNHFSSFKYSGNAVVESYSVLGSCRPSDPYSMSSVYSYHSRYAQPGLASVNGFHSKYTLPSFGYYGFPSSNPVFPSQFLGPSAWGHGGSGGSFEKKPDLHALHNSLNPAYGGAEFAELPGQAVATDNHHPIPHHQQPAYPGPKEYLLPKVPQLHPASRDPSPFAQSSSCYNRSIKQEPIDPLTQAESIPRDSAKMSRTPLPEASQNGGPSHLWGQYSGGPSMSPKRTNSVGGNWGVFPPGESPTIVPDKLNSFGASCLTPSHFPESQWGLFTGEGQQSAPHAGARLRGKPWSPCKFGNGTSALTGPSLTEKPWGMGTGDFNPALKGGPGFQDKLWNPVKVEEGRIPTPGANPLDKAWQAFGMPLSSNEKLFGALKSEEKLWDPFSLEEGTAEEPPSKGVVKEEKSGPTVEEDEEELWSDSEHNFLDENIGGVAVAPAHCSILIECARRELHATTPLKKPNRCHPTRISLVFYQHKNLNQPNHGLALWEAKMKQLAERARQRQEEAARLGLGQQEAKLYGKKRKWGGAMVAEPQHKEKKGAIPTRQALAMPTDSAVTVSSYAYTKVTGPYSRWI

SEQ ID NO: 3 - protein, 1795 aa, Homo sapiens
  source 1..1795: note = Human (homo sapiens) TET3-enzyme (Uniprot No O43151)
MSQFQVPLAVQPDLPGLYDFPQRQVMVGSFPGSGLSMAGSESQLRGGGDGRKKRKRCGTCEPCRRLENCGACTSCTNRRTHQICKLRKCEVLKKKVGLLKEVEIKAGEGAGPWGQGAAVKTGSELSPVDGPVPGQMDSGPVYHGDSRQLSASGVPVNGAREPAGPSLLGTGGPWRVDQKPDWEAAPGPAHTARLEDAHDLVAFSAVAEAVSSYGALSTRLYETFNREMSREAGNNSRGPRPGPEGCSAGSEDLDTLQTALALARHGMKPPNCNCDGPECPDYLEWLEGKIKSVVMEGGEERPRLPGPLPPGEAGLPAPSTRPLLSSEVPQISPQEGLPLSQSALSIAKEKNISLQTAIAIEALTQLSSALPQPSHSTPQASCPLPEALSPPAPFRSPQSYLRAPSWPVVPPEEHSSFAPDSSAFPPATPRTEFPEAWGTDTPPATPRSSWPMPRPSPDPMAELEQLLGSASDYIQSVFKRPEALPTKPKVKVEAPSSSPAPAPSPVLQREAPTPSSEPDTHQKAQTALQQHLHHKRSLFLEQVHDTSFPAPSEPSAPGWWPPPSSPVPRLPDRPPKEKKKKLPTPAGGPVGTEKAAPGIKPSVRKPIQIKKSRPREAQPLFPPVRQIVLEGLRSPASQEVQAHPPAPLPASQGSAVPLPPEPSLALFAPSPSRDSLLPPTQEMRSPSPMTALQPGSTGPLPPADDKLEELIRQFEAEFGDSFGLPGPPSVPIQDPENQQTCLPAPESPFATRSPKQIKIESSGAVTVLSTTCFHSEEGGQEATPTKAENPLTPTLSGFLESPLKYLDTPTKSLLDTPAKRAQAEFPTCDCVEQIVEKDEGPYYTHLGSGPTVASIRELMEERYGEKGKAIRIEKVIYTGKEGKSSRGCPIAKWVIRRHTLEEKLLCLVRHRAGHHCQNAVIVILILAWEGIPRSLGDTLYQELTDTLRKYGNPTSRRCGLNDDRTCACQGKDPNTCGASFSFGCSWSMYFNGCKYARSKTPRKFRLAGDNPKEEEVLRKSFQDLATEVAPLYKRLAPQAYQNQVTNEEIAIDCRLGLKEGRPFAGVTACMDFCAHAHKDQHNLYNGCTVVCTLTKEDNRCVGKIPEDEQLHVLPLYKMANTDEFGSEENQNAKVGSGAIQVLTAFPREVRRLPEPAKSCRQRQLEARKAAAEKKKIQKEKLSTPEKIKQEALELAGITSDPGLSLKGGLSQQGLKPSLKVEPQNHFSSFKYSGNAVVESYSVLGNCRPSDPYSMNSVYSYHSYYAQPSLTSVNGFHSKYALPSFSYYGFPSSNPVFPSQFLGPGAWGHSGSSGSFEKKPDLHALHNSLSPAYGGAEFAELPSQAVPTDAHHPTPHHQQPAYPGPKEYLLPKAPLLHSVSRDPSPFAQSSNCYNRSIKQEPVDPLTQAEPVPRDAGKMGKTPLSEVSQNGGPSHLWGQYSGGPSMSPKRTNGVGGSWGVFSSGESPAIVPDKLSSFGASCLAPSHFTDGQWGLFPGEGQQAASHSGGRLRGKPWSPCKFGNSTSALAGPSLTEKPWALGAGDFNSALKGSPGFQDKLWNPMKGEEGRIPAAGASQLDRAWQSFGLPLGSSEKLFGALKSEEKLWDPFSLEEGPAEEPPSKGAVKEEKGGGGAEEEEEELWSDSEHNFLDENIGGVAVAPAHGSILIECARRELHATTPLKKPNRCHPTRISLVFYQHKNLNQPNHGLALWEAKMKQLAERARARQEEAARLGLGQQEAKLYGKKRKWGGTVVAEPQQKEKKGVVPTRQALAVPTDSAVTVSSYAYTKVTGPYSRWI

SEQ ID NO: 4 - protein, 1901 aa, Xenopus tropicalis
  source 1..1901: note = Frog (Xenopus tropicalis) TET3-enzyme (Uniprot No A0JP82)
MDTQPAPVPHVLPQDVYEFPDDQESLGRLRVSEMPAELNGGGGGGSAAAFAMELPEQSNKKRKRCGVCVPCLRKEPCGACYNCVNRSTSHQICKMRKCEQLKKKRVVPMKGVENCSESILVDGPKTDQMEAGPVNHVQEGRLKQECDSTLPSKGCEDLANQLLMEANSWLSNTAAPQDPCNKLNWDKPTIPNHAANNNSNLEDAKNLVAFSAVAEAMSTYGMPASGTPSSVSLQLYEKFNYETNRDNSGHLEGNAPSCPEDLNTLKAALALAKHGVKPPNCNCDGPECPDYLEWLENKIKSTVKGSQESPFPNLGQVSKELVQKQYPKEQVLNLENKNSTCPSGNLPFSQNALSLAKEKNISLQTAIAIEALTQLSSALPQTNNECPNAPSQPLINPHDQLTHFPSAKGNQLPMLPVARNELFQNQQSQLYTGKNALPVPQSPRQTSWEQNKKSSYQEGQYIPENLSHSSSVLPSDASTPQKPEFLQQWVQNADLLKSPSDPMTGLKQLLGNTDEYIKSVFKGPEALPNKKNVKPKHTIKSIKKESTEFLKMSPDQQLSQLLQTNEFHRNTQAALQQHLHHKRNLFVDPNAMEACTQEQQNWWVPSSQQAPVSKTTEKPVKERKKRRQSPSQKQVEPKPKPQRKQVQIKKPKVKEGSAVFMPVSQISLDTFRRVEKEENQGKEMDAENSLPNNVQTELLESQSLQLTGSQANPDDRKTVNTQEMCNENQSNIGKANNFALCVNRANSFVAKDQCPTPSTHDTSSSSGQGDSANQHTNVSDVPGQNDLSCLDDKLEDLIRQFEAEFGEDFSLPGSAVPSQNGEGPPKQTPSGDPQFKLPFPSQLLPPENSTKPATHSNPALSNNPVSREVSNNLDSLFSSKSPKQIKIESSGAITVVSTTCFYSEENQHLDGTPTKSDLPFNPTLSGFLDSPLKYLTSPTKSLIDTPAKKAQAEFPTCDCVEQINEKDEGPYYTHLGSGPTVASIRELMEERFGQKGDAIRIEKVIYTGKEGKSSRGCPIAKWVIRRQSEDEKLMCLVRQRAGHHCENAVIIILIMAWEGIPRSLGDSLYNDITETITKYGNPTSRRCGLNDDRTCACQGKDPNTCGASFSFGCSWSMYFNGCKYARSKTPRKFRLIGENPKEEDGLKDNFQNLATKVAPVYKMLAPQAYQNQVNNEDIAIDCRLGLKEGRPFSGVTACMDFCAHAHKDQHNLYNGCTVVCTLTKEDNRMIGRVAEDEQLHVLPLYKVSTTDEFGSEEGQLEKIKKGGIHVLSSFPREVRKLSEPAKSCRQRQLEAKKAAAEKKKLQKEKLVSPDKTKQEPSDKKTCQQNPGVPQQQTKPCIKVEPSNHYNNFKYNGNGVVESYSVLGSCRPSDPYSMNSVYSYHSFYAQPNLPSVNGFHSKYALPPFGFYGFPNNPVVPNQFMNYGTSDARNSGWMNNCFEKKPELQSLADGMNQSYGSELSEQSFRRSSEVPHHYSLQNPSSQKSVNVPHRTTPAPVETTPYSNLPCYNKVIKKEPGSDPLVDSFQRANSVHSHSPGVNHSLQASDLPISYKANGALSSSGRTNAESPCSMFMPNDKNGLEKKDYFGVHSNAPGLKDKQWPPYGTDVSVRQHDSLDSQSPGKVWSSCKLSDSSAALPSSASTQDKNWNGRQVSLNQGMKESALFQEKLWNSVAASDRCSATPSDRSSITPCSELQDKNWGSFPNPTVNSLKTDSSQNHWDPYSLDDNMDDGQSKSVKEEDDEEIWSDSEHNFLDENIGGVAVAPGHGSILIECARRELHATTPLKKPNRCHPTRISLVFYQHKNLNQPNHGLALWEAKMKQLAERARAREEEAAKLGIKQEVKSLGKKRKWGGAATTETPPVEKKDYTPTRQAATILTDSATTSFSYAYTKVTGPYSRFI

SEQ ID NO: 5 - protein, 5 aa, synthetic construct
  source 1..5: note = C-terminal extension sequence of domain (a)
IQKEK

SEQ ID NO: 6 - protein, 5 aa, synthetic construct
  source 1..5: note = C-terminal extension sequence of domain (a)
LQKEK

SEQ ID NO: 7 - protein, 5 aa, synthetic construct
  source 1..5: note = C-terminal extension sequence of domain (b)
AARLG

SEQ ID NO: 8 - protein, 15 aa, synthetic construct
  source 1..15: note = connecting domain
GGGGSGGGGSGGGGS

SEQ ID NO: 9 - protein, 15 aa, synthetic construct
  source 1..15: note = connecting domain
GGGGSGGGGSGGGGE

SEQ ID NO: 10 - protein, 15 aa, synthetic construct
  source 1..15: note = connecting domain
GGGGSGGGGSGGGGD

SEQ ID NO: 11 - protein, 11 aa, synthetic construct
  source 1..11: note = Strep-tag II
MASWSHPQFEK

SEQ ID NO: 12 - protein, 13 aa, synthetic construct
  source 1..13: note = TEV protease cleavage site
SGGGGGENLYFQG

SEQ ID NO: 13 - protein, 16 aa, synthetic construct
  source 1..16: note = PreScission protease cleavage site
SGGGGGGALEVLFQGP

SEQ ID NO: 14 - protein, 353 aa, synthetic construct
  source 1..353: note = domain (a) of Mus musculus, amino acids 697-1048 of Uniprot No A0A5K1VVP6
SEFPTCDCVEQIVEKDEGPYYTHLGSGPTVASIRELMEDRYGEKGKAIRIEKVIYTGKEGKSSRGCPIAKWVIRRHTLEEKLLCLVRHRAGHHCQNAVIVILILAWEGIPRSLGDTLYQELTDTLRKYGNPTSRRCGLNDDRTCACQGKDPNTCGASFSFGCSWSMYFNGCKYARSKTPRKFRLTGDNPKEEEVLRNSFQDLATEVAPLYKRLAPQAYQNQVTNEDVAIDCRLGLKEGRPFSGVTACMDFCAHAHKDQHNLYNGCTVVCTLTKEDNRCVGQIPEDEQLHVLPLYKMASTDEFGSEENQNAKVSSGAIQVLTAFPREVRRLPEPAKSCRQRQLEARKAAAEKKK

SEQ ID NO: 15 - protein, 353 aa, synthetic construct; identical to SEQ ID NO: 14
  source 1..353: note = domain (a) of Mus musculus, amino acids 832-1183 of Uniprot No Q8BG87

SEQ ID NO: 16 - protein, 352 aa, synthetic construct
  source 1..352: note = domain (a) of Homo sapiens, amino acids 824-1175 of Uniprot No O43151
EFPTCDCVEQIVEKDEGPYYTHLGSGPTVASIRELMEERYGEKGKAIRIEKVIYTGKEGKSSRGCPIAKWVIRRHTLEEKLLCLVRHRAGHHCQNAVIVILILAWEGIPRSLGDTLYQELTDTLRKYGNPTSRRCGLNDDRTCACQGKDPNTCGASFSFGCSWSMYFNGCKYARSKTPRKFRLAGDNPKEEEVLRKSFQDLATEVAPLYKRLAPQAYQNQVTNEEIAIDCRLGLKEGRPFAGVAACMDFCAHAHKDQHNLYNGCTVVCTLTKEDNRCVGKIPEDEQLHVLPLYKMANTDEFGSEENQNAKVGSGAIQVLTAFPREVRRLPEPAKSCRQRQLEARKAAAEKKK

SEQ ID NO: 17 - protein, 352 aa, synthetic construct
  source 1..352: note = domain (a) of Xenopus tropicalis, amino acids 952-1304 of Uniprot No A0JP82
EFPTCDCVEQINEKDEGPYYTHLGSGPTVASIRELMEERFGQKGDAIRIEKVIYTGKEGKSSRGCPIAKWVIRRQSEDEKLMCLVRQRAGHHCENAVIIILIMAWEGIPRSLGDSLYNDITETITKYGNPTSRRCGLNDDRTCACQGKDPNTCGASFSFGCSWSMYFNGCKYARSKTPRKFRLIGENPKEEDGLKDNFQNLATKVAPVYKMLAPQAYQNQVNNEDIAIDCRLGLKEGRPFSGVTACMDFCAHAHKDQHNLYNGCTVVCTLTKEDNRMIGRVAEDEQLHVLPLYKVSTTDEFGSEEGQLEKIKKGGIHVLSSFPREVRKLSEPAKSCRQRQLEAKKAAAEKKK

SEQ ID NO: 18 - protein, 91 aa, synthetic construct
  source 1..91: note = domain (b) of Mus musculus, amino acids 1509-1599 Uniprot No A0A5K1VVP6
EELWSDSEHNFLDENIGGVAVAPAHCSILIECARRELHATTPLKKPNRCHPTRISLVFYQHKNLNQPNHGLALWEAKMKQLAERARQRQEE

SEQ ID NO: 19 - protein, 91 aa, synthetic construct; identical to SEQ ID NO: 18
  source 1..91: note = domain (b) of Mus musculus, amino acids 1643-1734 of Uniprot No Q8BG87

SEQ ID NO: 20 - protein, 92 aa, synthetic construct
  source 1..92: note = domain (b) of Homo sapiens, amino acids 1636-1726 of Uniprot No O43151
EEELWSDSEHNFLDENIGGVAVAPAHGSILIECARRELHATTPLKKPNRCHPTRISLVFYQHKNLNQPNHGLALWEAKMKQLAERARARQEE

SEQ ID NO: 21 - protein, 92 aa, synthetic construct
  source 1..92: note = domain (b) of Xenopus tropicalis, amino acids 1743-1833 of Uniprot No A0JP82
DEEIWSDSEHNFLDENIGGVAVAPGHGSILIECARRELHATTPLKKPNRCHPTRISLVFYQHKNLNQPNHGLALWEAKMKQLAERARAREEE